European Patent Specification EP 3 575 314 B1, published February 14, 2024. Title: Glucagon Derivatives With Improved Stability. Applicant: HANMI PHARM. CO., LTD. The sequence listing filed with the application follows.

SEQUENCE LISTING (36 sequences)

SEQ ID NO: 1 - protein, 29 aa, Homo sapiens
HSQGTFTSDYSKYLDSRRAQDFVQWLMNT

SEQ ID NO: 2 - protein, 29 aa, Artificial Sequence
  glucagon derivative
HSQGTFTSDYSKYLDCDRAQDFVQWLMNT

SEQ ID NO: 3 - protein, 29 aa, Artificial Sequence
  glucagon derivative
HSQGTFTSDYSKYLDCERAQDFVQWLMNT

SEQ ID NO: 4 - protein, 29 aa, Artificial Sequence
  glucagon derivative
HSQGTFTSDYSKYLDSCDAQDFVQWLMNT

SEQ ID NO: 5 - protein, 29 aa, Artificial Sequence
  glucagon derivative
HSQGTFTSDYSKYLDSCEAQDFVQWLMNT

SEQ ID NO: 6 - protein, 29 aa, Artificial Sequence
  glucagon derivative
HSQGTFTSDYSKYLDSCEADDFVQWLMNT

SEQ ID NO: 7 - protein, 29 aa, Artificial Sequence
  glucagon derivative
YSQGTFTSDYSKYLDSCEADDFVQWLMNT

SEQ ID NO: 8 - protein, 29 aa, Artificial Sequence
  glucagon derivative
  VARIANT (2): Xaa is aminoisobutyric acid
YXQGTFTSDYSKYLDSCDAQDFVQWLINT

SEQ ID NO: 9 - protein, 29 aa, Artificial Sequence
  glucagon derivative
  VARIANT (2): Xaa is aminoisobutyric acid
YXQGTFTSDYSKYLDSCDAQDFVVWLINT

SEQ ID NO: 10 - protein, 29 aa, Artificial Sequence
  glucagon derivative
  VARIANT (2): Xaa is aminoisobutyric acid
YXQGTFTSDYSKYLDSCDADDFVVWLINT

SEQ ID NO: 11 - protein, 29 aa, Artificial Sequence
  glucagon derivative
  VARIANT (2): Xaa is aminoisobutyric acid
YXQGTFTSDYSKYLDEKCAKEFVQWLMNT

SEQ ID NO: 12 - protein, 29 aa, Artificial Sequence
  glucagon derivative
  VARIANT (2): Xaa is aminoisobutyric acid
YXQGTFTSDYSKYLDSRRAQDFVQWLMNT

SEQ ID NO: 13 - protein, 29 aa, Artificial Sequence
  glucagon derivative
  VARIANT (2): Xaa is aminoisobutyric acid
YXQGTFTSDYSCYLDEKRAKEFVQWLMNT

SEQ ID NO: 14 - protein, 29 aa, Artificial Sequence
  glucagon derivative
  VARIANT (2): Xaa is aminoisobutyric acid
YXQGTFTSDYSKYLDCKRAKEFVQWLMNT

SEQ ID NO: 15 - protein, 29 aa, Artificial Sequence
  glucagon derivative
  VARIANT (2): Xaa is aminoisobutyric acid
YXQGTFTSDYSKYLCEKRAQDFVVWLMNT

SEQ ID NO: 16 - protein, 29 aa, Artificial Sequence
  glucagon derivative
  VARIANT (2): Xaa is aminoisobutyric acid
YXQGTFTSDYSKYLDCRRAQVFVQWLMRT

SEQ ID NO: 17 - protein, 29 aa, Artificial Sequence
  glucagon derivative
  VARIANT (2): Xaa is aminoisobutyric acid
YXQGTFTSDYSKYLDCVRAQDFVQWLMRT

SEQ ID NO: 18 - protein, 29 aa, Artificial Sequence
  glucagon derivative
  VARIANT (2): Xaa is aminoisobutyric acid
YXQGTFTSDYSKYLDSRRACDFRLWLMNT

SEQ ID NO: 19 - protein, 29 aa, Artificial Sequence
  glucagon derivative
  VARIANT (2): Xaa is aminoisobutyric acid
  VARIANT (16), (20): amino acids at position 16 and position 20 form a ring
YXQGTFTSDYSKYLCEKRAKEFVQWLMNT

SEQ ID NO: 20 - protein, 29 aa, Artificial Sequence
  glucagon derivative
  VARIANT (2): Xaa is aminoisobutyric acid
  VARIANT (16), (20): amino acids at position 16 and position 20 form a ring
YXQGTFTSDYSKYLDECRAKEFVQWLMNT

SEQ ID NO: 21 - protein, 29 aa, Artificial Sequence
  glucagon derivative
  VARIANT (2): Xaa is aminoisobutyric acid
  VARIANT (16), (20): amino acids at position 16 and position 20 form a ring
YXQGTFTSDYSKYLDEKCAKEFVQWLMNT

SEQ ID NO: 22 - protein, 29 aa, Artificial Sequence
  glucagon derivative
  VARIANT (2): Xaa is aminoisobutyric acid
  VARIANT (16), (20): amino acids at position 16 and position 20 form a ring
YXQGTFTSDYSKYLDEKRCKEFVQWLMNT

SEQ ID NO: 23 - protein, 29 aa, Artificial Sequence
  glucagon derivative
  VARIANT (2): Xaa is aminoisobutyric acid
  VARIANT (16), (20): amino acids at position 16 and position 20 form a ring
YXQGTFTSDYSKYCDEKRAKEFVQWLMNT

SEQ ID NO: 24 - protein, 29 aa, Artificial Sequence
  glucagon derivative
  VARIANT (2): Xaa is aminoisobutyric acid
  VARIANT (16), (20): amino acids at position 16 and position 20 form a ring
YXQGTFTSDYSKCLDEKRAKEFVQWLMNT

SEQ ID NO: 25 - protein, 29 aa, Artificial Sequence
  glucagon derivative
  VARIANT (2): Xaa is aminoisobutyric acid
  VARIANT (16), (20): amino acids at position 16 and position 20 form a ring
YXQGTFTSDYSKYLDEKRAKCFVQWLMNT

SEQ ID NO: 26 - protein, 29 aa, Artificial Sequence
  glucagon derivative
  VARIANT (2): Xaa is aminoisobutyric acid
  VARIANT (16), (20): amino acids at position 16 and position 20 form a ring
WXQGTFTSDYSKYLDECRAKDFVQWLMNT

SEQ ID NO: 27 - protein, 29 aa, Artificial Sequence
  glucagon derivative
  VARIANT (2): Xaa is aminoisobutyric acid
  VARIANT (16), (20): amino acids at position 16 and position 20 form a ring
YXQGTFVSDYSKYLDECRAKDFVQWLMNT

SEQ ID NO: 28 - protein, 29 aa, Artificial Sequence
  glucagon derivative
  VARIANT (2): Xaa is aminoisobutyric acid
  VARIANT (16), (20): amino acids at position 16 and position 20 form a ring
WXQGTFVSDYSKYLDECRAKDFVQWLMNT

SEQ ID NO: 29 - protein, 29 aa, Artificial Sequence
  glucagon derivative
  VARIANT (2): Xaa is aminoisobutyric acid
  VARIANT (16), (20): amino acids at position 16 and position 20 form a ring
YXQGTFTSDYSKCLDERRAKDFVQWLMNT

SEQ ID NO: 30 - protein, 29 aa, Artificial Sequence
  glucagon derivative
  VARIANT (2): Xaa is aminoisobutyric acid
  VARIANT (16), (20): amino acids at position 16 and position 20 form a ring
WXQGTFTSDYSKCLDERRAEDFVQWLMNT

SEQ ID NO: 31 - protein, 29 aa, Artificial Sequence
  glucagon derivative
  VARIANT (2): Xaa is aminoisobutyric acid
  VARIANT (17), (21): amino acids at position 17 and position 21 form a ring
YXQGTFTSDYSKYLDCKRAKEFVQWLMNT

SEQ ID NO: 32 - protein, 28 aa, Artificial Sequence
  glucagon derivative
  VARIANT (15), (19): amino acids at position 15 and position 19 form a ring
SQGTFTSDYSKYLDECRAKEFVQWLMNT

SEQ ID NO: 33 - protein, 29 aa, Artificial Sequence
  glucagon derivative
  VARIANT (2): Xaa is aminoisobutyric acid
  VARIANT (16), (20): amino acids at position 16 and position 20 form a ring
WXQGTFTSDYSKYCDERRAKEFVQWLMNT

SEQ ID NO: 34 - protein, 29 aa, Artificial Sequence
  glucagon derivative
  VARIANT (2): Xaa is aminoisobutyric acid
  VARIANT (16), (20): amino acids at position 16 and position 20 form a ring
YXQGTFTSDYSKYCDERRAKEFVQWLMNT

SEQ ID NO: 35 - DNA, 34 bp, Artificial Sequence
  forward primer
cagcgacaccgaccgtccccccgtacttaaggcc

SEQ ID NO: 36 - DNA, 32 bp, Artificial Sequence
  reverse primer
ctaaccgactctcggggaagactgagctcgcc